European Patent Application EP 4 692 123 A1, published February 11, 2026. Title: ANTI-BCAM ANTIBODY AND ANTIBODY-DRUG CONJUGATE. Applicant: GENOME AND COMPANY. The sequence listing filed with the application follows.

SEQUENCE LISTING (8 sequences)

SEQ ID NO: 1 - protein, 118 aa, synthetic construct
EVQLVESGGGLVKPGGSLRLSCAASGFTFSSYSMNWVRQAPGKGLEWVSSISSSSSYIYYADSVKGRFTISRDNAKNSLYLQMNSLRAEDTAVYYCARIIGGWLGDYWGQGTLVTVSS

SEQ ID NO: 2 - protein, 108 aa, synthetic construct
NIQMTQSPSSVSASVGDRVTITCRASQGISSWLAWYQQKPGKAPKLLIYAASSLRSGVPSRFSGSGSGTDFTLTISSLQPEDFATYYCQQANSFPPPTFGGGTKVEIK

SEQ ID NO: 3 - protein, 10 aa, synthetic construct
GFTFSSYSMN

SEQ ID NO: 4 - protein, 17 aa, synthetic construct
SISSSSSYIYYADSVKG

SEQ ID NO: 5 - protein, 11 aa, synthetic construct
ARIIGGWLGDY

SEQ ID NO: 6 - protein, 11 aa, synthetic construct
RASQGISSWLA

SEQ ID NO: 7 - protein, 7 aa, synthetic construct
AASSLRS

SEQ ID NO: 8 - protein, 10 aa, synthetic construct
QQANSFPPPT